European Patent Application EP 4 755 913 A1, published June 10, 2026. Title: EGFR/c-Met双特异性抗体及其应用. Applicant: 白先宏. Application WO, filed July 13, 2024. The sequence listing filed with the application follows.

SEQUENCE LISTING (34 sequences)

SEQ ID NO: 1 - protein, 219 aa, synthetic construct
DIQMTQSPSSLSASVGDRVTITCRSSQNIVHSNGNTYLDWYQQTPGKAPKLLIYKVSNRFSGVPSRFSGSGSGTDFTFTISSLQPEDIATYYCFQYSHVPWTFGQGTKLQITRTVAAPSVFIFPPSDEQLKSGTASVVCLLNNFYPREAKVQWKVDNALQSGNSQESVTEQDSKDSTYSLSSTLTLSKADYEKHKVYACEVTHQGLSSPVTKSFNRGEC

SEQ ID NO: 2 - protein, 453 aa, synthetic construct
QVQLQQSGAEVKKPGSSVKVSCKASGYTFTNYYIYWVRQAPGQGLEWIGGINPTSGGSNFNEKFKTRVTITADESSTTAYMELSSLRSEDTAFYFCTRQGLWFDSDGRGFDFWGQGTTVTVSSASTKGPSVFPLAPSSKSTSGGTAALGCLVKDYFPEPVTVSWNSGALTSGVHTFPAVLQSSGLYSLSSVVTVPSSSLGTQTYICNVNHKPSNTKVDKRVEPKSCDKTHTCPPCPAPELLGGPSVFLFPPKPKDTLMISRTPEVTCVVVDVSHEDPEVKFNWYVDGVEVHNAKTKPREEQYNSTYRVVSVLTVLHQDWLNGKEYKCKVSNKALPAPIEKTISKAKGQPREPQVYTLPPSREEMTKNQVSLTCLVKGFYPSDIAVEWESNGQPENNYKTTPPVLDSDGSFLLYSKLTVDKSRWQQGNVFSCSVMHEALHNHYTQKSLSLSPGK

SEQ ID NO: 3 - protein, 215 aa, synthetic construct
DIQMTQSPSSLSASVGDRVTITCSVSSSVSSIYLHWYQQKPGKAPKLLIYSTSNLASGVPSRFSGSGSGTDFTLTISSLQPEDFATYYCQVYSGYPLTFGGGTKVEIKRTVAAPSVFIFPPSDEQLKSGTASVVCLLNNFYPREAKVQWKVDNALQSGNSQESVTEQDSKDSTYSLSSTLTLSKADYEKHKVYACEVTHQGLSSPVTKSFNRGEC

SEQ ID NO: 4 - protein, 445 aa, synthetic construct
QVQLVQSGAEVKKPGASVKVSCKASGYTFTDYYMHWVRQAPGQGLEWMGRVNPNRRGTTYNQKFEGRVTMTTDTSTSTAYMELRSLRSDDTAVYYCARANWLDYWGQGTTVTVSSASTKGPSVFPLAPSSKSTSGGTAALGCLVKDYFPEPVTVSWNSGALTSGVHTFPAVLQSSGLYSLSSVVTVPSSSLGTQTYICNVNHKPSNTKVDKRVEPKSCDKTHTCPPCPAPELLGGPSVFLFPPKPKDTLMISRTPEVTCVVVDVSHEDPEVKFNWYVDGVEVHNAKTKPREEQYNSTYRVVSVLTVLHQDWLNGKEYKCKVSNKALPAPIEKTISKAKGQPREPQVYTLPPSREEMTKNQVSLTCLVKGFYPSDIAVEWESNGQPENNYKTTPPVLDSDGSFFLYSRLTVDKSRWQQGNVFSCSVMHEALHNHYTQKSLSLSPGK

SEQ ID NO: 5 - protein, 123 aa, synthetic construct [sequence omitted]

SEQ ID NO: 6 - protein, 112 aa, synthetic construct [sequence omitted]

SEQ ID NO: 7 - protein, 115 aa, synthetic construct [sequence omitted]

SEQ ID NO: 8 - protein, 108 aa, synthetic construct [sequence omitted]

SEQ ID NO: 9 - protein, 232 aa, synthetic construct
EPKSCDKTHTCPPCPAPELLGGPSVFLFPPKPKDTLMISRTPEVTCVVVDVSHEDPEVKFNWYVDGVEVHNAKTKPREEQYNSTYRVVSVLTVLHQDWLNGKEYKCKVSNKALPAPIEKTISKAKGQPREPQVYTLPPSREEMTKNQVSLTCLVKGFYPSDIAVEWESNGQPENNYKTTPPVLDSDGSFLLYSKLTVDKSRWQQGNVFSCSVMHEALHNHYTQKSLSLSPGK

SEQ ID NO: 10 - protein, 232 aa, synthetic construct
EPKSCDKTHTCPPCPAPELLGGPSVFLFPPKPKDTLMISRTPEVTCVVVDVSHEDPEVKFNWYVDGVEVHNAKTKPREEQYNSTYRVVSVLTVLHQDWLNGKEYKCKVSNKALPAPIEKTISKAKGQPREPQVYTLPPSREEMTKNQVSLTCLVKGFYPSDIAVEWESNGQPENNYKTTPPVLDSDGSFFLYSRLTVDKSRWQQGNVFSCSVMHEALHNHYTQKSLSLSPGK

SEQ ID NO: 11 - protein, 330 aa, synthetic construct
ASTKGPSVFPLAPSSKSTSGGTAALGCLVKDYFPEPVTVSWNSGALTSGVHTFPAVLQSSGLYSLSSVVTVPSSSLGTQTYICNVNHKPSNTKVDKRVEPKSCDKTHTCPPCPAPELLGGPSVFLFPPKPKDTLMISRTPEVTCVVVDVSHEDPEVKFNWYVDGVEVHNAKTKPREEQYNSTYRVVSVLTVLHQDWLNGKEYKCKVSNKALPAPIEKTISKAKGQPREPQVYTLPPSREEMTKNQVSLTCLVKGFYPSDIAVEWESNGQPENNYKTTPPVLDSDGSFLLYSKLTVDKSRWQQGNVFSCSVMHEALHNHYTQKSLSLSPGK

SEQ ID NO: 12 - protein, 107 aa, synthetic construct [sequence omitted]

SEQ ID NO: 13 - protein, 330 aa, synthetic construct
ASTKGPSVFPLAPSSKSTSGGTAALGCLVKDYFPEPVTVSWNSGALTSGVHTFPAVLQSSGLYSLSSVVTVPSSSLGTQTYICNVNHKPSNTKVDKRVEPKSCDKTHTCPPCPAPELLGGPSVFLFPPKPKDTLMISRTPEVTCVVVDVSHEDPEVKFNWYVDGVEVHNAKTKPREEQYNSTYRVVSVLTVLHQDWLNGKEYKCKVSNKALPAPIEKTISKAKGQPREPQVYTLPPSREEMTKNQVSLTCLVKGFYPSDIAVEWESNGQPENNYKTTPPVLDSDGSFFLYSRLTVDKSRWQQGNVFSCSVMHEALHNHYTQKSLSLSPGK

SEQ ID NO: 14 - protein, 107 aa, synthetic construct [sequence omitted]

SEQ ID NO: 15 - DNA, 1359 bp, synthetic construct
  source 1..1359: mol_type = other DNA
caagtccaactccagcagagtggtgccgaagtgaaaaagcctggcagctctgtcaaagtctcctgtaaggcttcaggctacactttcaccaactactacatctactgggtgcggcaggctcctggtcagggcttggaatggataggcggtatcaaccctacaagtggaggttcaaacttcaacgagaagttcaagacccgcgttacaatcactgctgacgagagcagcaccacagcttatatggaactcagttccctgcggtctgaagacacagccttctatttctgcacacggcaggggctttggtttgatagtgacggtcgagggtttgacttctggggacaaggcactactgtaacagtgtcttcagcctccactaaaggcccatccgtgttccctctggctccaagtagcaagtccactagcggagggacagctgcactgggttgccttgttaaggattatttccccgaacccgtcacagtctcttggaatagtggcgccctcacttccggcgtccataccttcccagctgtgctgcagtcctctgggctctacagcctgagcagcgtcgttactgtcccatctagcagtctgggaacccaaacatacatatgtaacgtcaatcacaagccttctaacacaaaagtggacaagagggtagagcccaagagttgtgacaaaacacatacatgtcctccatgcccagctcctgaacttcttggaggcccatctgttttcctgtttccccctaagccaaaagacaccttgatgatttctcgtacccccgaagtcacctgcgttgtggtggacgtatcacacgaggaccccgaagtcaagttcaactggtatgtggatggcgtcgaagtccacaacgctaagacaaaaccccgtgaggagcagtacaacagtacctatagggtggtcagtgtgcttaccgtgcttcaccaagattggcttaatgggaaggagtacaaatgcaaggtgtccaacaaagcactgccagcaccaatcgagaagactatcagtaaagctaaggggcagcccagggagcctcaagtgtatacccttccccctagccgggaggagatgacaaagaaccaagtgagcttgacatgcctcgtgaaaggattttatccttccgacatagcagtggagtgggaaagtaatgggcagcccgaaaacaactataagaccaccccacctgttttggatagcgatggcagttttctgctttactctaagctgaccgttgataaaagtagatggcagcagggcaacgttttcagttgctccgtgatgcatgaagcactccacaatcactatacacagaaatccctgagcctgtctccaggcaaa

SEQ ID NO: 16 - DNA, 657 bp, synthetic construct
  source 1..657: mol_type = other DNA
gatatccagatgactcagagtccaagttctctgtcagcctccgtgggcgatcgagtgaccattacttgcagatcatcccagaacatcgtccactctaatgggaatacctacctggactggtatcaacagaccccagggaaggccccaaagctcctgatctacaaggtgtccaacaggtttagcggtgtgccaagcagattctcagggagtggttctggcactgattttaccttcactatctcctccttgcagcccgaagacatcgccacttattattgtttccagtattcccacgtgccttggacctttggccaggggactaagctgcaaattactcgaacagtggctgccccttccgtctttatcttccccccttcagatgagcagctgaaatccggaactgccagtgtagtgtgcctgctgaataacttctaccctagagaggcaaaggtccagtggaaggtggacaatgcccttcaaagcggaaactctcaggaatcagtcacagagcaggactccaaggatagtacctattctctttcttcaacactgactctgagtaaagccgattacgagaagcacaaagtctatgcatgtgaagtgactcatcagggactgtctagtccagttactaaatcttttaacaggggggaatgt

SEQ ID NO: 17 - DNA, 1335 bp, synthetic construct
  source 1..1335: mol_type = other DNA
caagtgcaattggtgcaatctggcgctgaagttaaaaaaccaggagcaagtgttaaagtatcttgtaaggcctccggctatacctttacagactactatatgcattgggtcagacaagctccaggtcagggcctggaatggatgggaagagtgaacccaaatcggcgtggaaccacatacaatcagaaattcgaggggagagttaccatgaccaccgacacctcaacctctaccgcttatatggagctgcgaagtctccggtctgatgataccgctgtgtactattgcgccagagccaactggctcgactattggggccagggcactactgtcacagtgagcagtgcctccactaagggaccctccgtctttcctctggctccttcctccaagtcaacatcaggtggcacagctgctctgggatgtttggtgaaggattatttccccgagcctgttaccgtgagttggaactcaggtgctctcacttctggggtgcatacatttcccgccgtcctgcagtcttccggattgtatagcctgtcaagtgtggtcaccgtgccctctagttccctgggaacacagacatacatttgcaacgtgaatcacaagcccagcaatactaaggtggacaagagggttgaacccaagagttgcgataaaacacatacttgtcctccctgtcctgcaccagagctgcttgggggaccaagtgtattcctttttccccccaagcctaaggacactctgatgatcagccggactcctgaggtgacctgtgtagtggtagacgtttcacatgaggatcccgaagtgaagttcaactggtatgtggatggggttgaagtgcataatgcaaagacaaaaccacgagaggaacagtacaattccacttatagggtcgtttcagtgctgaccgttctgcaccaggactggctgaacggtaaagagtataaatgcaaggtgtccaataaggctctgcctgctcctatcgaaaagactattagcaaggctaaagggcagcctagagaaccacaggtctatactctcccccccagccgtgaggagatgactaaaaatcaggtgagcctcacatgcctggtgaagggcttctacccctcagatatcgcagtggaatgggaaagcaatggacagcccgagaacaactacaaaaccacacctccagttttggattctgacgggtctttctttctgtacagcaggttgaccgtggataagagccgatggcagcaagggaacgtgttttcttgctccgtgatgcacgaggccctgcacaatcactacacacaaaagtccctgtccctgagcccaggcaaa

SEQ ID NO: 18 - DNA, 645 bp, synthetic construct
  source 1..645: mol_type = other DNA
gatattcagatgactcagtccccaagctccttgtccgcctccgttggtgaccgggtcaccatcacatgctccgtatcctcctccgtctcctctatctatttgcactggtatcagcagaagcccggtaaagccccaaaactgctcatctatagtacaagcaatctggccagtggagtgccttctcgctttagcggcagcggctcaggaaccgattttacactgaccatctcctccctgcagcccgaagatttcgccacatattattgtcaggtgtactccggatatccacttaccttcggtggcgggacaaaagtggagataaaacggactgtggccgcaccatccgttttcatctttcccccctccgacgaacaactcaagtccggcacagcttctgtggtgtgcctgctgaataacttctacccaagggaggccaaagtccagtggaaagtggacaacgctctgcagagcggcaattctcaggaatctgtgactgagcaggattcaaaagattctacttacagtctgtcctccaccctgacactctccaaggccgactatgagaaacacaaggtgtacgcatgcgaggtaactcaccagggactgtccagtcctgttacaaagtcctttaatcgtggcgaatgt

SEQ ID NO: 19 - protein, 5 aa, synthetic construct
NYYIY

SEQ ID NO: 20 - protein, 17 aa, synthetic construct
GINPTSGGSNFNEKFKT

SEQ ID NO: 21 - protein, 14 aa, synthetic construct
QGLWFDSDGRGFDF

SEQ ID NO: 22 - protein, 16 aa, synthetic construct
RSSQNIVHSNGNTYLD

SEQ ID NO: 23 - protein, 7 aa, synthetic construct
KVSNRFS

SEQ ID NO: 24 - protein, 9 aa, synthetic construct
FQYSHVPWT

SEQ ID NO: 25 - protein, 5 aa, synthetic construct
DYYMH

SEQ ID NO: 26 - protein, 17 aa, synthetic construct
RVNPNRRGTTYNQKFEG

SEQ ID NO: 27 - protein, 6 aa, synthetic construct
ANWLDY

SEQ ID NO: 28 - protein, 12 aa, synthetic construct
SVSSSVSSIYLH

SEQ ID NO: 29 - protein, 7 aa, synthetic construct
STSNLAS

SEQ ID NO: 30 - protein, 9 aa, synthetic construct
QVYSGYPLT

SEQ ID NO: 31 - protein, 908 aa, synthetic construct
ECKEALAKSEMNVNMKYQLPNFTAETPIQNVILHEHHIFLGATNYIYVLNEEDLQKVAEYKTGPVLEHPDCFPCQDCSSKANLSGGVWKDNINMALVVDTYYDDQLISCGSVNRGTCQRHVFPHNHTADIQSEVHCIFSPQIEEPSQCPDCVVSALGAKVLSSVKDRFINFFVGNTINSSYFPDHPLHSISVRRLKETKDGFMFLTDQSYIDVLPEFRDSYPIKYVHAFESNNFIYFLTVQRETLDAQTFHTRIIRFCSINSGLHSYMEMPLECILTEKRKKRSTKKEVFNILQAAYVSKPGAQLARQIGASLNDDILFGVFAQSKPDSAEPMDRSAMCAFPIKYVNDFFNKIVNKNNVRCLQHFYGPNHEHCFNRTLLRNSSGCEARRDEYRTEFTTALQRVDLFMGQFSEVLLTSISTFIKGDLTIANLGTSEGRFMQVVVSRSGPSTPHVNFLLDSHPVSPEVIVEHTLNQNGYTLVITGKKITKIPLNGLGCRHFQSCSQCLSAPPFVQCGWCHDKCVRSEECLSGTWTQQICLPAIYKVFPNSAPLEGGTRLTICGWDFGFRRNNKFDLKKTRVLLGNESCTLTLSESTMNTLKCTVGPAMNKHFNMSIIISNGHGTTQYSTFSYVDPVITSISPKYGPMAGGTLLTLTGNYLNSGNSRHISIGGKTCTLKSVSNSILECYTPAQTISTEFAVKLKIDLANRETSIFSYREDPIVYEIHPTKSFISGGSTITGVGKNLNSVSVPRMVINVHEAGRNFTVACQHRSNSEIICCTTPSLQQLNLQLPLKTKAFFMLDGILSKYFDLIYVHNPVFKPFEKPVMISMGNENVLEIKGNDIDPEAVKGEVLKVGNKSCENIHLHSEAVLCTVPNDLLKLNSELNIEWKQAISSTVLGKVIVQPDQNFT

SEQ ID NO: 32 - protein, 621 aa, synthetic construct [sequence omitted]

SEQ ID NO: 33 - protein, 107 aa, synthetic construct
GQPREPQVYTLPPSREEMTKNQVSLTCLVKGFYPSDIAVEWESNGQPENNYKTTPPVLDSDGSFLLYSKLTVDKSRWQQGNVFSCSVMHEALHNHYTQKSLSLSPGK

SEQ ID NO: 34 - protein, 107 aa, synthetic construct
GQPREPQVYTLPPSREEMTKNQVSLTCLVKGFYPSDIAVEWESNGQPENNYKTTPPVLDSDGSFFLYSRLTVDKSRWQQGNVFSCSVMHEALHNHYTQKSLSLSPGK